European Patent Application EP 4 656 632 A1, published December 3, 2025. Title: Novel diagnostic fluorescent probe for fire blight bacteria. Applicant: University-Industry Cooperation Group of Kyung Hee University. The sequence listing filed with the application follows.

SEQUENCE LISTING (2 sequences)

SEQ ID NO: 1 - DNA, 28 bp, synthetic construct
  source 1..28: mol_type = other DNA; note = Forward primer
gcactgaggtttttagggatatccgctg

SEQ ID NO: 2 - DNA, 28 bp, synthetic construct
  source 1..28: mol_type = other DNA; note = Reverse primer
gctcaatcgccagggaaatgatatcggc